European Patent Application EP 4 365 292 A1, published May 8, 2024. Title: Aptamer for the detection of the microorganism Bacillus subtilis. Applicant: CONSIGLIO PER LA RICERCA IN AGRICOLTURA E L'ANALISI DELL'ECONOMIA AGRARIA. The sequence listing filed with the application follows.

SEQUENCE LISTING (7 sequences)

SEQ ID NO: 1 - DNA, 20 bp, synthetic construct
  source 1..20: mol_type = other DNA
aagtgagcgaagcggttacg

SEQ ID NO: 2 - DNA, 22 bp, synthetic construct
  source 1..22: mol_type = other DNA
agttgacatctgcgatgctgat

SEQ ID NO: 3 - DNA, 24 bp, Bacillus subtilis
  source 1..24: mol_type = genomic DNA
ctacccctcttttgagaaggccga

SEQ ID NO: 4 - DNA, 25 bp, Bacillus subtilis
  source 1..25: mol_type = genomic DNA
cctcttttgagaaggccgatcacca

SEQ ID NO: 5 - DNA, 21 bp, Bacillus subtilis
  source 1..21: mol_type = genomic DNA
cgatcagcatcgcagatgtca

SEQ ID NO: 6 - DNA, 23 bp, Bacillus subtilis
  source 1..23: mol_type = genomic DNA
cgatcagcatcgcagatgtcaac

SEQ ID NO: 7 - DNA, 19 bp, Bacillus subtilis
  source 1..19: mol_type = genomic DNA
cctcttttgagaaggccga